European Patent Application EP 4 119 659 A1, published January 18, 2023. Title: Mannanase variants. Applicant: AB Enzymes. The sequence listing filed with the application follows.

SEQUENCE LISTING (1 sequence)

SEQ ID NO: 1 - protein, 414 aa, Artificial Sequence
  Variant parent
VSTPVNGYVLERVVILSRHGVRSPTKQTDLMNNVTPDKWPQWPVQAGYLTPQGEHLMTLMGGFYRDYFRSHNLLPSQGCPTDGSLYVWADIDQRTRLTGQAFLAGVAPECDLKIHHQADLKTTDALFHPVEAGICKLDKQQTQQAVEKQLGAPLATLSQRYALPLAQMGEILNFAASPYCKEMQTKGQSCDFASFTPNQIHLSPNGQKVSLSGPLALSSTLSEIFLLQYAQGMPEVAWQRLSGEDNWRSLMSLHNEQFNLMAKTPYIASHKGTPLLKEISATLAGQQGTLKRPANNRILFIAGHDTNIANIAGMLGLNWELPHQPDNTPPGGGLVFELWNNPQDHQQYVSVKMFYQTMEQLRNGEKLDMHHPAGMVQVAIAGCENSNSSVLCSLKDLQKKVSQAIQPACQLSMQ